European Patent Specification EP 3 540 066 B1, published December 24, 2025. Title: Common Light Chain Mouse. Applicant: BUCKLER, David R. MCWHIRTER, John MACDONALD, Lynn STEVENS, Sean DAVIS, Samuel MURPHY, Andrew J. Application To be assigned. The sequence listing filed with the application follows.

SEQUENCE LISTING (18 sequences)

SEQ ID NO: 1 - DNA, 3155 bp, Artificial Sequence
  Synthetic
ggcgcgccgtagctttgaattttaaacatctatttgacaagaaatgcatagttccttctctttaaaataatgtaatgtttctttcaagaataagcttggtttgatgcctctctccccaacatgatagaagtgtagcataaatctatgaaaaattccatttccctgtgcctacaacaactacctgggattgaaaacttcttcccttgctctagtcctttcttctacacctacttccacatcatctgtgactcaaaacaatacttgtcaggaaagatcccggaaagagcaaaaaagacttccttagaggtgtcagagattcctatgccactatctgtcatctctagaaggggttgtgagtatgaggaagagcagagcttgtaaattttctacttgctttgacttccactgtatttcctaacaacaacaaccacagcaacacccataacatcacaggacaaacttctagtacttccaaggctttagtctcagtaaatcttctctacctccatcacagcagctagaaggtttgatactcatacaaatagtactgtagctttctgttcataattggaaaaatagacaagacccaatgtaatacaggctttccttcagccagttagcgttcagtttttggatcaccattgcacacatatacccagcatatgtctaatatatatgtagaaatccgtgaagcaagagttataatagcttgtgttttctattgtattgtattttcctcttatatcatcttcttcttcgttcattaaaaaaaaaccgttcaagtaggtctaaattaattattggatcataagtagataaaatattttatttcataacacattgacccgatgaatatgtttctttgccagacatagtcctcatttccaaggtaacaagcctgaaaaaattatactggagcaagtcaacaggtaatgatggtagcttttccttattgtcctggggcaagaataagacaaaagataacagggtagaataaagattgtgtaagaaagaaggacagcaacaggacatgggaaccttttatagagtaacattttgataatggatgatgagaattaatgagttagacagggatgggtgggaatgattgaaggtgtgagtactttagcacagattaagaccaaatcattaggatttaaagagttgtgtagagttagtgaaggaaaagccttagaattaaatttggctgcggataaaacattcttggattagactgaagactcttttctgtgctaagtaagtatatttatgataatgatgatgactgtagtgctgaatatttaataaataaaaacaaaattaattgccgcatacataatgtcctgaatactattgtaaatgttttatcttatttcctttaaactgtctacagcactataaggtaggtaccagtattgtcacagttacacagatatggaaaccgagacacagggaagttaagttacttgatcaatttcaagcaatcggcaagccatggagcatctatgtcagggctgccaggacatgtgactgtaaacagaagtttttcactttttaactcaaagagggtatgtggctgggttaatggaaagcttcaggaccctcagaaaacattactaacaagcaaatgaaaggtgtatctggaagattaagttttaacagactcttcatttccatcgatccaataatgcacttagggagatgactgggcatattgaggataggaagagagaagtgaaaacacagctttttatattgttcttaacaggcttgtgccaaacatcttctgggtggatttaggtgattgaggagaagaaagacacaggagcgaaattctctgagcacaagggaggagttctacactcagactgagccaacagacttttctggcctgacaaccagggcggcgcaggatgctcagtgcagagaggaagaagcaggtggtctttgcagctgaaagctcagctgatttgcatatggagtcattatacaacatcccagaattctttaagggcagctgccaggaagctaagaagcatcctctcttctagctctcagagatggagacagacacactcctgctatgggtgctgctgctctgggttccaggtgagggtacagataagtgttatgagcaacctctgtggccattatgatgctccatgcctctctgttcttgatcactataattagggcatttgtcactggttttaagtttccccagtcccctgaattttccattttctcagagtgatgtccaaaattattcttaaaaatttaaatgaaaaggtcctctgctgtgaaggcttttaaagatatataaaaataatctttgtgtttatcattccaggtgccagatgtgacatccagatgacccagtctccatcctccctgtctgcatctgtaggagacagagtcaccatcacttgccgggcaagtcagagcattagcagctatttaaattggtatcagcagaaaccagggaaagcccctaagctcctgatctatgctgcatccagtttgcaaagtggggtcccatcaaggttcagtggcagtggatctgggacagatttcactctcaccatcagcagtctgcaacctgaagattttgcaacttactactgtcaacagagttacagtacccctccgatcaccttcggccaagggacacgactggagattaaacgtaagtaatttttcactattgtcttctgaaatttgggtctgatggccagtattgacttttagaggcttaaataggagtttggtaaagattggtaaatgagggcatttaagatttgccatgggttgcaaaagttaaactcagcttcaaaaatggatttggagaaaaaaagattaaattgctctaaactgaatgacacaaagtaaaaaaaaaaagtgtaactaaaaaggaacccttgtatttctaaggagcaaaagtaaatttatttttgttcactcttgccaaatattgtattggttgttgctgattatgcatgatacagaaaagtggaaaaatacattttttagtctttctcccttttgtttgataaattattttgtcagacaacaataaaaatcaatagcacgccctaagatctagatgcatgctcgagtgccatttcattacctctttctccgcacccgacatagat

SEQ ID NO: 2 - DNA, 28 bp, Artificial Sequence
  Synthetic
aggtgagggtacagataagtgttatgag

SEQ ID NO: 3 - DNA, 27 bp, Artificial Sequence
  Synthetic
tgacaaatgccctaattatagtgatca

SEQ ID NO: 4 - DNA, 21 bp, Artificial Sequence
  Synthetic
gggcaagtcagagcattagca

SEQ ID NO: 5 - DNA, 21 bp, Artificial Sequence
  Synthetic
tgcaaactggatgcagcatag

SEQ ID NO: 6 - DNA, 19 bp, Artificial Sequence
  Synthetic
ggtggagaggctattcggc

SEQ ID NO: 7 - DNA, 17 bp, Artificial Sequence
  Synthetic
gaacacggcggcatcag

SEQ ID NO: 8 - DNA, 23 bp, Artificial Sequence
  Synthetic
tgggcacaacagacaatcggctg

SEQ ID NO: 9 - DNA, 29 bp, Artificial Sequence
  Synthetic
ccattatgatgctccatgcctctctgttc

SEQ ID NO: 10 - DNA, 26 bp, Artificial Sequence
  Synthetic
atcagcagaaaccagggaaagcccct

SEQ ID NO: 11 - DNA, 3166 bp, Artificial Sequence
  Synthetic
ggcgcgccgtagctttgaattttaaacatctatttgacaagaaatgcatagttccttctctttaaaataatgtaatgtttctttcaagaataagcttggtttgatgcctctctccccaacatgatagaagtgtagcataaatctatgaaaaattccatttccctgtgcctacaacaactacctgggattgaaaacttcttcccttgctctagtcctttcttctacacctacttccacatcatctgtgactcaaaacaatacttgtcaggaaagatcccggaaagagcaaaaaagacttccttagaggtgtcagagattcctatgccactatctgtcatctctagaaggggttgtgagtatgaggaagagcagagcttgtaaattttctacttgctttgacttccactgtatttcctaacaacaacaaccacagcaacacccataacatcacaggacaaacttctagtacttccaaggctttagtctcagtaaatcttctctacctccatcacagcagctagaaggtttgatactcatacaaatagtactgtagctttctgttcataattggaaaaatagacaagacccaatgtaatacaggctttccttcagccagttagcgttcagtttttggatcaccattgcacacatatacccagcatatgtctaatatatatgtagaaatccgtgaagcaagagttataatagcttgtgttttctattgtattgtattttcctcttatatcatcttcttcttcgttcattaaaaaaaaaccgttcaagtaggtctaaattaattattggatcataagtagataaaatattttatttcataacacattgacccgatgaatatgtttctttgccagacatagtcctcatttccaaggtaacaagcctgaaaaaattatactggagcaagtcaacaggtaatgatggtagcttttccttattgtcctggggcaagaataagacaaaagataacagggtagaataaagattgtgtaagaaagaaggacagcaacaggacatgggaaccttttatagagtaacattttgataatggatgatgagaattaatgagttagacagggatgggtgggaatgattgaaggtgtgagtactttagcacagattaagaccaaatcattaggatttaaagagttgtgtagagttagtgaaggaaaagccttagaattaaatttggctgcggataaaacattcttggattagactgaagactcttttctgtgctaagtaagtatatttatgataatgatgatgactgtagtgctgaatatttaataaataaaaacaaaattaattgccgcatacataatgtcctgaatactattgtaaatgttttatcttatttcctttaaactgtctacagcactataaggtaggtaccagtattgtcacagttacacagatatggaaaccgagacacagggaagttaagttacttgatcaatttcaagcaatcggcaagccatggagcatctatgtcagggctgccaggacatgtgactgtaaacagaagtttttcactttttaactcaaagagggtatgtggctgggttaatggaaagcttcaggaccctcagaaaacattactaacaagcaaatgaaaggtgtatctggaagattaagttttaacagactcttcatttccatcgatccaataatgcacttagggagatgactgggcatattgaggataggaagagagaagtgaaaacacagctttttatattgttcttaacaggcttgtgccaaacatcttctgggtggatttaggtgattgaggagaagaaagacacaggagcgaaattctctgagcacaagggaggagttctacactcagactgagccaacagacttttctggcctgacaaccagggcggcgcaggatgctcagtgcagagaggaagaagcaggtggtctttgcagctgaaagctcagctgatttgcatatggagtcattatacaacatcccagaattctttaagggcagctgccaggaagctaagaagcatcctctcttctagctctcagagatggagacagacacactcctgctatgggtgctgctgctctgggttccaggtgagggtacagataagtgttatgagcaacctctgtggccattatgatgctccatgcctctctgttcttgatcactataattagggcatttgtcactggttttaagtttccccagtcccctgaattttccattttctcagagtgatgtccaaaattattcttaaaaatttaaatgaaaaggtcctctgctgtgaaggcttttaaagatatataaaaataatctttgtgtttatcattccaggtgccagatgtataccaccggagaaattgtgttgacgcagtctccaggcaccctgtctttgtctccaggggaaagagccaccctctcctgcagggccagtcagagtgttagcagcagctacttagcctggtaccagcagaaacctggccaggctcccaggctcctcatctatggtgcatccagcagggccactggcatcccagacaggttcagtggcagtgggtctgggacagacttcactctcaccatcagcagactggagcctgaagattttgcagtgtattactgtcagcagtatggtagctcaccttggacgttcggccaagggaccaaggtggaaatcaaacgtaagtaatttttcactattgtcttctgaaatttgggtctgatggccagtattgacttttagaggcttaaataggagtttggtaaagattggtaaatgagggcatttaagatttgccatgggttgcaaaagttaaactcagcttcaaaaatggatttggagaaaaaaagattaaattgctctaaactgaatgacacaaagtaaaaaaaaaaagtgtaactaaaaaggaacccttgtatttctaaggagcaaaagtaaatttatttttgttcactcttgccaaatattgtattggttgttgctgattatgcatgatacagaaaagtggaaaaatacattttttagtctttctcccttttgtttgataaattattttgtcagacaacaataaaaatcaatagcacgccctaagatctagatgcatgctcgagtgccatttcattacctctttctccgcacccgacatagat

SEQ ID NO: 12 - DNA, 19 bp, Artificial Sequence
  Synthetic
tccaggcaccctgtctttg

SEQ ID NO: 13 - DNA, 26 bp, Artificial Sequence
  Synthetic
aagtagctgctgctaacactctgact

SEQ ID NO: 14 - DNA, 24 bp, Artificial Sequence
  Synthetic
aaagagccaccctctcctgcaggg

SEQ ID NO: 15 - DNA, 3187 bp, Artificial Sequence
  Synthetic
ggcgcgccgtagctttgaattttaaacatctatttgacaagaaatgcatagttccttctctttaaaataatgtaatgtttctttcaagaataagcttggtttgatgcctctctccccaacatgatagaagtgtagcataaatctatgaaaaattccatttccctgtgcctacaacaactacctgggattgaaaacttcttcccttgctctagtcctttcttctacacctacttccacatcatctgtgactcaaaacaatacttgtcaggaaagatcccggaaagagcaaaaaagacttccttagaggtgtcagagattcctatgccactatctgtcatctctagaaggggttgtgagtatgaggaagagcagagcttgtaaattttctacttgctttgacttccactgtatttcctaacaacaacaaccacagcaacacccataacatcacaggacaaacttctagtacttccaaggctttagtctcagtaaatcttctctacctccatcacagcagctagaaggtttgatactcatacaaatagtactgtagctttctgttcataattggaaaaatagacaagacccaatgtaatacaggctttccttcagccagttagcgttcagtttttggatcaccattgcacacatatacccagcatatgtctaatatatatgtagaaatccgtgaagcaagagttataatagcttgtgttttctattgtattgtattttcctcttatatcatcttcttcttcgttcattaaaaaaaaaccgttcaagtaggtctaaattaattattggatcataagtagataaaatattttatttcataacacattgacccgatgaatatgtttctttgccagacatagtcctcatttccaaggtaacaagcctgaaaaaattatactggagcaagtcaacaggtaatgatggtagcttttccttattgtcctggggcaagaataagacaaaagataacagggtagaataaagattgtgtaagaaagaaggacagcaacaggacatgggaaccttttatagagtaacattttgataatggatgatgagaattaatgagttagacagggatgggtgggaatgattgaaggtgtgagtactttagcacagattaagaccaaatcattaggatttaaagagttgtgtagagttagtgaaggaaaagccttagaattaaatttggctgcggataaaacattcttggattagactgaagactcttttctgtgctaagtaagtatatttatgataatgatgatgactgtagtgctgaatatttaataaataaaaacaaaattaattgccgcatacataatgtcctgaatactattgtaaatgttttatcttatttcctttaaactgtctacagcactataaggtaggtaccagtattgtcacagttacacagatatggaaaccgagacacagggaagttaagttacttgatcaatttcaagcaatcggcaagccatggagcatctatgtcagggctgccaggacatgtgactgtaaacagaagtttttcactttttaactcaaagagggtatgtggctgggttaatggaaagcttcaggaccctcagaaaacattactaacaagcaaatgaaaggtgtatctggaagattaagttttaacagactcttcatttccatcgatccaataatgcacttagggagatgactgggcatattgaggataggaagagagaagtgaaaacacagctttttatattgttcttaacaggcttgtgccaaacatcttctgggtggatttaggtgattgaggagaagaaagacacaggagcgaaattctctgagcacaagggaggagttctacactcagactgagccaacagacttttctggcctgacaaccagggcggcgcaggatgctcagtgcagagaggaagaagcaggtggtctttgcagctgaaagctcagctgatttgcatatggagtcattatacaacatcccagaattctttaagggcagctgccaggaagctaagaagcatcctctcttctagctctcagagatggagacagacacactcctgctatgggtgctgctgctctgggttccaggtgagggtacagataagtgttatgagcaacctctgtggccattatgatgctccatgcctctctgttcttgatcactataattagggcatttgtcactggttttaagtttccccagtcccctgaattttccattttctcagagtgatgtccaaaattattcttaaaaatttaaatgaaaaggtcctctgctgtgaaggcttttaaagatatataaaaataatctttgtgtttatcattccaggtgccagatgtgttgtggtcctcagccggtgctgcatcagccgccggccatgtcctcggcccttggaaccacaatccgcctcacctgcaccctgaggaacgaccatgacatcggtgtgtacagcgtctactggtaccagcagaggccgggccaccctcccaggttcctgctgagatatttctcacaatcagacaagagccagggcccccaggtcccccctcgcttctctggatccaaagatgtggccaggaacagggggtatttgagcatctctgagctgcagcctgaggacgaggctatgtattactgtgctatgcataactcagtgacgcatgtgtttggcagcgggacccagctcaccgttttaagtaagtaatttttcactattgtcttctgaaatttgggtctgatggccagtattgacttttagaggcttaaataggagtttggtaaagattggtaaatgagggcatttaagatttgccatgggttgcaaaagttaaactcagcttcaaaaatggatttggagaaaaaaagattaaattgctctaaactgaatgacacaaagtaaaaaaaaaaagtgtaactaaaaaggaacccttgtatttctaaggagcaaaagtaaatttatttttgttcactcttgccaaatattgtattggttgttgctgattatgcatgatacagaaaagtggaaaaatacattttttagtctttctcccttttgtttgataaattattttgtcagacaacaataaaaatcaatagcacgccctaagatctagatgcatgctcgagtgccatttcattacctctttctccgcacccgacatagat

SEQ ID NO: 16 - DNA, 17 bp, Artificial Sequence
  Synthetic
tgtcctcggcccttgga

SEQ ID NO: 17 - DNA, 20 bp, Artificial Sequence
  Synthetic
ccgatgtcatggtcgttcct

SEQ ID NO: 18 - DNA, 23 bp, Artificial Sequence
  Synthetic
acaatccgcctcacctgcaccct